European Patent Specification EP 3 837 283 B1, published April 17, 2024. Title: Anti-IL1RAP antibody compositions. Applicant: Cantargia AB. Application PCT/EP2019/071974. The sequence listing filed with the application follows.

SEQUENCE LISTING (38 sequences)

SEQ ID NO: 1 - protein, 108 aa, Synthetic
  CAN04 variant 6 variable light chain (VL)
DIQMTQSPSSLSASVGDRVTITCQASQGINNYLNWYQQKPGKAPKLLIHYTSGLHAGVPSRFSGSGSGTDYTLTISSLEPEDVATYYCQQYSILPWTFGGGTKVEIKR

SEQ ID NO: 2 - protein, 108 aa, Synthetic
  CAN04 variable light chain (VL) VL1
DIQMTQSPSSLSASVGDRVTITCSASQGINNYLNWYQQKPGKAPKLLIHYTSGLHAGVPSRFSGSGSGTDYTLTISSLQPEDVATYYCQQYSILPWTFGGGTKVEIKR

SEQ ID NO: 3 - protein, 108 aa, Synthetic
  CAN04 variable light chain (VL) VL3
DIQMTQSPSSLSASVGDRVTITCQASQGINNYLNWYQQKPGKAPKLLIHYTSGLHAGVPSRFSGSGSGTDFTLTISSLEPEDVATYYCQQYSILPWTFGGGTKVEIKR

SEQ ID NO: 4 - protein, 117 aa, Synthetic
  CAN04 variant 6 variable heavy chain (VH)
QVQLVQSGAEVKKPGSSVKVSCKASGYAFTSSWMNWVRQAPGQGLEWMGRIYPGDGNTHYAQKFQGRVTLTADKSTSTAYMELSSLRSEDTAVYYCGEGYLDPMDYWGQGTLVTVSS

SEQ ID NO: 5 - protein, 117 aa, Synthetic
  CAN04 variable heavy chain (VH) VH1
QVQLVQSGAEVKKPGSSVKVSCKASGYAFSSSWMNWVRQAPGQGLEWMGRIYPGDGNTHYAQKFQGRVTLTADKSTSTAYMELSSLRSEDTAVYYCGEGYLDPMDYWGQGTLVTVSS

SEQ ID NO: 6 - protein, 117 aa, Synthetic
  CAN04 variable heavy chain (VH) VH3
QVQLVQSGAEVKKPGSSVKVSCKASGYTFTSSWMNWVRQAPGKGLEWMGRIYPGDGQTHYAQKFQGRVTLTADKSTSTAYMELSSLRSEDTAVYYCGEGYLDPMDYWGQGTLVTVSS

SEQ ID NO: 7 - protein, 117 aa, Synthetic
  CAN04 variable heavy chain (VH) VH4
QVQLVQSGAEVKKPGSSVKVSCKASGYTFTSSWMNWVRQAPGKGLEWMGRIYPGDGQTHYAQKFQGRVTITADKSTSTAYMELSSLRSEDTAVYYCGEGYLDPMDYWGQGTLVTVSS

SEQ ID NO: 8 - protein, 11 aa, Synthetic
  CAN04 variant 6 Light chain CDR1 (according to Chotia)
SASQGINNYLN

SEQ ID NO: 9 - protein, 9 aa, Synthetic
  CAN04 variant 6 Light chain CDR2 (according to Chotia)
YTSGLHAGV

SEQ ID NO: 10 - protein, 9 aa, Synthetic
  CAN04 variant 6 Light chain CDR3 (according to Chotia)
QQYSILPWT

SEQ ID NO: 11 - protein, 11 aa, Synthetic
  CAN04 variant 6 Heavy chain CDR1 (according to Chotia)
GYAFTSSSWMN

SEQ ID NO: 12 - protein, 17 aa, Synthetic
  CAN04 variant 6 Heavy chain CDR2 (according to Chotia)
RIYPGDGNTHYAQKFQG

SEQ ID NO: 13 - protein, 8 aa, Synthetic
  CAN04 variant 6 Heavy chain CDR3 (according to Chotia)
GYLDPMDY

SEQ ID NO: 14 - protein, 108 aa, Synthetic
  CAN03 variable light chain (VL)
DILLTQSPAILSVSPGERVSFSCRASQSIGTSIHWYQRRTNGSPRLLIKSASESISGIPSRFSGSGSGTDFTLSINSVESEDIADYYCQQSNSWPTTFGAGTKLELKR

SEQ ID NO: 15 - protein, 119 aa, Synthetic
  CAN03 variable heavy chain (VH)
DVKLVESGGGLVKPGGSLKLSCAASGFTFSIYTMSWVRQTPEKRLEWVATISIGGSYINYPDSVKGRFTISRDNAKNTLYLQMSSLKSEDTAIYYCSREVDGSYAMDYWGQGTSVTVSS

SEQ ID NO: 16 - protein, 11 aa, Synthetic
  CAN03 Light chain CDR1 (according to Chotia)
RASQSIGTSIH

SEQ ID NO: 17 - protein, 7 aa, Synthetic
  CAN03 Light chain CDR2 (according to Chotia)
SASESIS

SEQ ID NO: 18 - protein, 9 aa, Synthetic
  CAN03 Light chain CDR3 (according to Chotia)
QQSNSWPTT

SEQ ID NO: 19 - protein, 10 aa, Synthetic
  CAN03 Heavy chain CDR1 (according to Chotia)
GFTFSIYTMS

SEQ ID NO: 20 - protein, 17 aa, Synthetic
  CAN03 Heavy chain CDR2 (according to Chotia)
TISIGGSYINYPDSVKG

SEQ ID NO: 21 - protein, 10 aa, Synthetic
  CAN03 Heavy chain CDR3 (according to Chotia)
EVDGSYAMDY

SEQ ID NO: 22 - protein, 7 aa, Synthetic
  CAN04 variant 6 Variable light chain CDR2 (according to Kabat)
YTSGLHA

SEQ ID NO: 23 - protein, 8 aa, Synthetic
  CAN04 variant 6 Variable light chain CDR3 (according to Kabat)
QYSILPWT

SEQ ID NO: 24 - protein, 7 aa, Synthetic
  CAN04 variant 6 Variable heavy chain CDR1 (according to Kabat)
GYAFTSS

SEQ ID NO: 25 - protein, 6 aa, Synthetic
  CAN04 variant 6 Variable heavy chain CDR2 (according to Kabat)
YPGDGN

SEQ ID NO: 26 - protein, 8 aa, Synthetic
  CAN03 Variable light chain CDR3 (according to Kabat)
QSNSWPTT

SEQ ID NO: 27 - protein, 7 aa, Synthetic
  CAN03 Variable heavy chain CDR1(according to Kabat)
GFTFSIY

SEQ ID NO: 28 - protein, 6 aa, Synthetic
  CAN03 Variable heavy chain CDR2 (according to Kabat)
SIGGSY

SEQ ID NO: 29 - protein, 10 aa, Synthetic
  CAN04 variant 6 Light chain CDR1 (according to Kabat)
ASQGINNYLN

SEQ ID NO: 30 - protein, 10 aa, Synthetic
  CAN03 Light chain CDR1 (according to Kabat)
ASQSIGTSIH

SEQ ID NO: 31 - protein, 329 aa, Synthetic
  CAN04 Heavy chain constant region
ASTKGPSVFPLAPSSKSTSGGTAALGCLVKDYFPEPVTVSWNSGALTSGVHTFPAVLQSSLYSLSSVVTVPSSSLGTQTYICNVNHKPSNTKVDKKVEPKSCDKTHTCPPCPAPELLGGPSVFLFPPKPKDTLMISRTPEVTCVVVDVSHEDPEVKFNWYVDGVEVHNAKTKPREEQYNSTYRVVSVLTVLHQDWLNGKEYKCKVSNKALPAPIEKTISKAKGQPREPQVYTLPPSREEMTKNQVSLTCLVKGFYPSDIAVEWESNGQPENNYKTTPPVLDSDGSFFLYSKLTVDKSRWQQGNVFSCSVMHEALHNHYTQKSLSLSPGK

SEQ ID NO: 32 - protein, 106 aa, Synthetic
  CAN04 Light chain constant region
TVAAPSVFIFPPSDEQLKSGTASVVCLLNNFYPREAKVQWKVDNALQSGNSQESVTEQDSKDSTYSLSSTLTLSKADYEKHKVYACEVTHQGLSSPVTKSFNRGEC

SEQ ID NO: 33 - protein, 320 aa, Homo sapiens
  CAN03 Heavy chain constant region, Ig gamma-1 chain C region (UnitProt Accession No. P01857)
ASTKGPSVFPLAPSSKSTSGGTAALGCLVKDYFPEPVTVSWNSGALTSGVHTFPAVLQSSGLYSLSSVVTVPSSSLGTQTYICNVNHKPSNTKVDKKVEPKSCDKTHTCPPCPAPELLGGPSVFLFPPKPKDTLMISRTPEVTCVVVDVSHEDPEVKFNWYVDGVEVHNAKTKPREEQYNSTYRVVSVLTVLHQDWLNGKEYKCKVSNKALPAPIEKTISKAKGQPREPQVYTLPPSREEMTKNQVSLTCLVKGFYPSDIAVEWESNGQPENNYKTTPPVLDSDGSFFLYSKLTVDKSRWQQGNVFSCSVMHEALHNHYT

SEQ ID NO: 34 - protein, 106 aa, Homo sapiens; identical to SEQ ID NO: 32
  CAN03 Light chain constant region, Ig kappa chain C region (UnitProt Accession No. P01834)

SEQ ID NO: 35 - protein, 447 aa, Synthetic
  hu3F8-HC-hIgG1-K409R
QVQLVQSGAEVKKPGSSVKVSCKASGYAFTSSWMNWVRQAPGQGLEWMGRIYPGDGNTHYAQKFQGRVTLTADKSTSTAYMELSSLRSEDTAVYYCGEGYLDPMDYWGQGTLVTVSSASTKGPSVFPLAPSSKSTSGGTAALGCLVKDYFPEPVTVSWNSGALTSGVHTFPAVLQSSGLYSLSSVVTVPSSSLGTQTYICNVNHKPSNTKVDKKVEPKSCDKTHTCPPCPAPELLGGPSVFLFPPKPKDTLMISRTPEVTCVVVDVSHEDPEVKFNWYVDGVEVHNAKTKPREEQYNSTYRVVSVLTVLHQDWLNGKEYKCKVSNKALPAPIEKTISKAKGQPREPQVYTLPPSREEMTKNQVSLTCLVKGFYPSDIAVEWESNGQPENNYKTTPPVLDSDGSFFLYSRLTVDKSRWQQGNVFSCSVMHEALHNHYTQKSLSLSPGK

SEQ ID NO: 36 - protein, 214 aa, Synthetic
  hu3F8-LC-hk
DIQMTQSPSSLSASVGDRVTITCQASQGINNYLNWYQQKPGKAPKLLIHYTSGLHAGVPSRFSGSGSGTDYTLTISSLEPEDVATYYCQQYSILPWTFGGGTKVEIKRTVAAPSVFIFPPSDEQLKSGTASVVCLLNNFYPREAKVQWKVDNALQSGNSQESVTEQDSKDSTYSLSSTLTLSKADYEKHKVYACEVTHQGLSSPVTKSFNRGEC

SEQ ID NO: 37 - protein, 449 aa, Synthetic
  ch2C9-HC-hIgG1-F405L
DVKLVESGGGLVKPGGSLKLSCAASGFTFSIYTMSWVRQTPEKRLEWVATISIGGSYINYPDSVKGRFTISRDNAKNTLYLQMSSLKSEDTAIYYCSREVDGSYAMDYWGQGTSVTVSSASTKGPSVFPLAPSSKSTSGGTAALGCLVKDYFPEPVTVSWNSGALTSGVHTFPAVLQSSGLYSLSSVVTVPSSSLGTQTYICNVNHKPSNTKVDKKVEPKSCDKTHTCPPCPAPELLGGPSVFLFPPKPKDTLMISRTPEVTCVVVDVSHEDPEVKFNWYVDGVEVHNAKTKPREEQYNSTYRVVSVLTVLHQDWLNGKEYKCKVSNKALPAPIEKTISKAKGQPREPQVYTLPPSREEMTKNQVSLTCLVKGFYPSDIAVEWESNGQPENNYKTTPPVLDSDGSFLLYSKLTVDKSRWQQGNVFSCSVMHEALHNHYTQKSLSLSPGK

SEQ ID NO: 38 - protein, 214 aa, Synthetic
  ch2C9-LC-hk
DILLTQSPAILSVSPGERVSFSCRASQSIGTSIHWYQRRTNGSPRLLIKSASESISGIPSRFSGSGSGTDFTLSINSVESEDIADYYCQQSNSWPTTFGAGTKLELKRTVAAPSVFIFPPSDEQLKSGTASVVCLLNNFYPREAKVQWKVDNALQSGNSQESVTEQDSKDSTYSLSSTLTLSKADYEKHKVYACEVTHQGLSSPVTKSFNRGEC